European Patent Application EP 4 610 352 A1, published September 3, 2025. Title: SERINE PROTEASE FOR SELECTIVELY DEGRADING MUCINS AND USE THEREOF. Applicant: Zhenglong Sun. Application EP. The sequence listing filed with the application follows.

SEQUENCE LISTING (3 sequences)

SEQ ID NO: 1 - protein, 1364 aa, Escherichia coli
MNKVFSLKYSFLAKGFIAVSELARRVSVKGKLKSASSIIISPITIAIVSYAPPSLAATVNADISYQTFRDFAENKGAFIVGASNINIYDKNGVLVGVLDKAPMPDFSSATMNTGTLPPGDHTLYSPQYVVTAKHVNGSDIMSFGHIQNNYTVVGENNHNSLDIKIRRLNKIVTEVAPAEISSVGAVNGAYQEGGRFKAFYRLGGGLQYIKDKNGNLTPVYTNGGFLTGGTISALSSYNNGQMITAPTGDIFNPANGPLANYLNKGDSGSPLFAYDSLDKKWVLVGVLSSGSEHGNNWVVTTQDFLHQQPKHDFDKTISYDSEKGSLQWRYNKNSGVGTLSQESVVWDMHGKKGGDLNAGKNLQFTGNNGEIILHDSIDQGAGYLQFFDNYTVTSLTDQTWTGGGIITEKGVNVLWQVNGVNDDNLHKVGEGTLTVNGKGVNNGGLKVGDGTVILNQRPDDNGHKQAFSSINISSGRATVILSDANQVNPDKISWGYRGGTLDLNGNNVNFTRLQAADYGAIVSNNNKNKSELTLKLQTLNENDISVDVKTYEVFGGHGSPGDLYYVPASNTYFILKSKAYGPFFSDLDNTNVWQNVGHDRDKAIQIVKQQKIGESSQPYMFHGQLNGYMDVNIHPLSGKDVLTLDGSVNLPEGVITKKSGTLIFQGHPVIHAGMTTSAGQSDWENRQFTMDKLRLDAATFHLSRNAHMQGDISAANGSTVILGSSRVFTDKNDGTGNAVSSVEGSSIATTAGDQSYYSGNVLLENHSSLEVRENFTGGIEAYDSSVSVTSQNAIFDHVGSFVNSSLLLEKGAKLTAQSGIFTNNTMKIKENASLTLTGIPSVGKPGYYSPVTSTTEGIHLGERASLSVKNMGYLSSNITAENSAAIINLGDSNATIGKTDSPLFSTLMRGYNAVLQGNIMGPQSSVNMNNALWHSDRNSELKELKANDSQIELGVRGHFAKLRVKELIASNSVFLVHANNSQADQLNVTDKLQGSNNTILVDFFNKAANGTNVTLITAPKGSDENTFKAGTQQIGFSNITPEIRTENTDTATQWVLTGYQSVADARASKIATDFMDSGYKSFLTEVNNLNKRMGDLRDSQGDAGGWARIMNGTGSGESGYRDNYTHVQIGADRKHELNGIDLFTGALLTYTDNNASSQAFSGKTKSLGGGVYASGLFESGAYFDLIGKYLHHDNRYTLNFASLGERSYTSHSLYAGAEIGYRYHMSENTWVEPQMELVYGSVSGKSFNWKDQGMQLSMKDKDYHPLIGRTGVDVGRAFSGDTWKVTVRAGLGYQFDLLANGETVLQDASGKKHFKGEKDSRMLMNVGTNVEVKDNMRFGLELEKSAFGRYNIDNSINANFRYYF

SEQ ID NO: 2 - protein, 1042 aa, Escherichia coli
ATVNADISYQTFRDFAENKGAFIVGASNINIYDKNGVLVGVLDKAPMPDFSSATMNTGTLPPGDHTLYSPQYVVTAKHVNGSDIMSFGHIQNNYTVVGENNHNSLDIKIRRLNKIVTEVAPAEISSVGAVNGAYQEGGRFKAFYRLGGGLQYIKDKNGNLTPVYTNGGFLTGGTISALSSYNNGQMITAPTGDIFNPANGPLANYLNKGDSGSPLFAYDSLDKKWVLVGVLSSGSEHGNNWVVTTQDFLHQQPKHDFDKTISYDSEKGSLQWRYNKNSGVGTLSQESVVWDMHGKKGGDLNAGKNLQFTGNNGEIILHDSIDQGAGYLQFFDNYTVTSLTDQTWTGGGIITEKGVNVLWQVNGVNDDNLHKVGEGTLTVNGKGVNNGGLKVGDGTVILNQRPDDNGHKQAFSSINISSGRATVILSDANQVNPDKISWGYRGGTLDLNGNNVNFTRLQAADYGAIVSNNNKNKSELTLKLQTLNENDISVDVKTYEVFGGHGSPGDLYYVPASNTYFILKSKAYGPFFSDLDNTNVWQNVGHDRDKAIQIVKQQKIGESSQPYMFHGQLNGYMDVNIHPLSGKDVLTLDGSVNLPEGVITKKSGTLIFQGHPVIHAGMTTSAGQSDWENRQFTMDKLRLDAATFHLSRNAHMQGDISAANGSTVILGSSRVFTDKNDGTGNAVSSVEGSSIATTAGDQSYYSGNVLLENHSSLEVRENFTGGIEAYDSSVSVTSQNAIFDHVGSFVNSSLLLEKGAKLTAQSGIFTNNTMKIKENASLTLTGIPSVGKPGYYSPVTSTTEGIHLGERASLSVKNMGYLSSNITAENSAAIINLGDSNATIGKTDSPLFSTLMRGYNAVLQGNIMGPQSSVNMNNALWHSDRNSELKELKANDSQIELGVRGHFAKLRVKELIASNSVFLVHANNSQADQLNVTDKLQGSNNTILVDFFNKAANGTNVTLITAPKGSDENTFKAGTQQIGFSNITPEIRTENTDTATQWVLTGYQSVADARASKIATDFMDSGYKSFLTEVNNLNKRMGDLRD

SEQ ID NO: 3 - protein, 1308 aa, Escherichia coli
ATVNADISYQTFRDFAENKGAFIVGASNINIYDKNGVLVGVLDKAPMPDFSSATMNTGTLPPGDHTLYSPQYVVTAKHVNGSDIMSFGHIQNNYTVVGENNHNSLDIKIRRLNKIVTEVAPAEISSVGAVNGAYQEGGRFKAFYRLGGGLQYIKDKNGNLTPVYTNGGFLTGGTISALSSYNNGQMITAPTGDIFNPANGPLANYLNKGDSGSPLFAYDSLDKKWVLVGVLSSGSEHGNNWVVTTQDFLHQQPKHDFDKTISYDSEKGSLQWRYNKNSGVGTLSQESVVWDMHGKKGGDLNAGKNLQFTGNNGEIILHDSIDQGAGYLQFFDNYTVTSLTDQTWTGGGIITEKGVNVLWQVNGVNDDNLHKVGEGTLTVNGKGVNNGGLKVGDGTVILNQRPDDNGHKQAFSSINISSGRATVILSDANQVNPDKISWGYRGGTLDLNGNNVNFTRLQAADYGAIVSNNNKNKSELTLKLQTLNENDISVDVKTYEVFGGHGSPGDLYYVPASNTYFILKSKAYGPFFSDLDNTNVWQNVGHDRDKAIQIVKQQKIGESSQPYMFHGQLNGYMDVNIHPLSGKDVLTLDGSVNLPEGVITKKSGTLIFQGHPVIHAGMTTSAGQSDWENRQFTMDKLRLDAATFHLSRNAHMQGDISAANGSTVILGSSRVFTDKNDGTGNAVSSVEGSSIATTAGDQSYYSGNVLLENHSSLEVRENFTGGIEAYDSSVSVTSQNAIFDHVGSFVNSSLLLEKGAKLTAQSGIFTNNTMKIKENASLTLTGIPSVGKPGYYSPVTSTTEGIHLGERASLSVKNMGYLSSNITAENSAAIINLGDSNATIGKTDSPLFSTLMRGYNAVLQGNIMGPQSSVNMNNALWHSDRNSELKELKANDSQIELGVRGHFAKLRVKELIASNSVFLVHANNSQADQLNVTDKLQGSNNTILVDFFNKAANGTNVTLITAPKGSDENTFKAGTQQIGFSNITPEIRTENTDTATQWVLTGYQSVADARASKIATDFMDSGYKSFLTEVNNLNKRMGDLRDSQGDAGGWARIMNGTGSGESGYRDNYTHVQIGADRKHELNGIDLFTGALLTYTDNNASSQAFSGKTKSLGGGVYASGLFESGAYFDLIGKYLHHDNRYTLNFASLGERSYTSHSLYAGAEIGYRYHMSENTWVEPQMELVYGSVSGKSFNWKDQGMQLSMKDKDYHPLIGRTGVDVGRAFSGDTWKVTVRAGLGYQFDLLANGETVLQDASGKKHFKGEKDSRMLMNVGTNVEVKDNMRFGLELEKSAFGRYNIDNSINANFRYYF